European Patent Application EP 4 342 972 A1, published March 27, 2024. Title: Immobilized extracellular vesicle for in vitro assays. Applicant: Max-Planck-Gesellschaft zur Forderung der Wissenschaften e.V. The sequence listing filed with the application follows.

SEQUENCE LISTING (24 sequences)

SEQ ID NO: 1 - DNA, 25 bp, synthetic construct
  source 1..25: mol_type = other DNA
ttatgcaagactggatttcctgaag

SEQ ID NO: 2 - DNA, 20 bp, synthetic construct
  source 1..20: mol_type = other DNA
cttgaaatctgctggctcgc

SEQ ID NO: 3 - DNA, 20 bp, synthetic construct
  source 1..20: mol_type = other DNA
tggccaccagtaacatgcaa

SEQ ID NO: 4 - DNA, 20 bp, synthetic construct
  source 1..20: mol_type = other DNA
gtcgttagcttcgtgcttgg

SEQ ID NO: 5 - DNA, 21 bp, synthetic construct
  source 1..21: mol_type = other DNA
gtgttcctacccccaatgtgt

SEQ ID NO: 6 - DNA, 24 bp, synthetic construct
  source 1..24: mol_type = other DNA
attgtcataccaggaaatgagctt

SEQ ID NO: 7 - DNA, 22 bp, synthetic construct
  source 1..22: mol_type = other DNA
cctcctgatagtgtggtgtctg

SEQ ID NO: 8 - DNA, 23 bp, synthetic construct
  source 1..23: mol_type = other DNA
cgtacacccagcttgaagccaat

SEQ ID NO: 9 - DNA, 19 bp, synthetic construct
  source 1..19: mol_type = other DNA
ggcgagtctgacatggctg

SEQ ID NO: 10 - DNA, 20 bp, synthetic construct
  source 1..20: mol_type = other DNA
gctggacgcagtgtcttctc

SEQ ID NO: 11 - DNA, 21 bp, synthetic construct
  source 1..21: mol_type = other DNA
tcttcctggtccccacagttt

SEQ ID NO: 12 - DNA, 23 bp, synthetic construct
  source 1..23: mol_type = other DNA
gcaagaatagttctcgggatgaa

SEQ ID NO: 13 - DNA, 19 bp, synthetic construct
  source 1..19: mol_type = other DNA
ccctgaagtcgaggagctg

SEQ ID NO: 14 - DNA, 19 bp, synthetic construct
  source 1..19: mol_type = other DNA
ctgctgcacctctaagcga

SEQ ID NO: 15 - DNA, 24 bp, synthetic construct
  source 1..24: mol_type = other DNA
atcggaccaggctcagaggtattg

SEQ ID NO: 16 - DNA, 22 bp, synthetic construct
  source 1..22: mol_type = other DNA
gttctcattgttgtcggcttcc

SEQ ID NO: 17 - DNA, 21 bp, synthetic construct
  source 1..21: mol_type = other DNA
taccagtgtctaccagccaat

SEQ ID NO: 18 - DNA, 21 bp, synthetic construct
  source 1..21: mol_type = other DNA
tgcacgagtatgaggaggtct

SEQ ID NO: 19 - DNA, 19 bp, synthetic construct
  source 1..19: mol_type = other DNA
gacagctacgcgcacatga

SEQ ID NO: 20 - DNA, 19 bp, synthetic construct
  source 1..19: mol_type = other DNA
ggtgcatcggttgcatctg

SEQ ID NO: 21 - DNA, 20 bp, synthetic construct
  source 1..20: mol_type = other DNA
gacattcccaaggaggaggc

SEQ ID NO: 22 - DNA, 20 bp, synthetic construct
  source 1..20: mol_type = other DNA
cttggtcttcaggtacgggg

SEQ ID NO: 23 - DNA, 20 bp, synthetic construct
  source 1..20: mol_type = other DNA
gcttctctggcacgtcttga

SEQ ID NO: 24 - DNA, 18 bp, synthetic construct
  source 1..18: mol_type = other DNA
cgcagggcatcgttgttc